European Patent Application EP 4 374 868 A1, published May 29, 2024. Title: 缓解或治疗纤维化性疾病的药物组合物或药盒及其应用. Applicant: 上海循曜生物科技有限公司. The sequence listing filed with the application follows.

SEQUENCE LISTING (109 sequences)

SEQ ID NO: 1 - protein, 117 aa, synthetic construct
EVQLQQSGPELVKPGASMKISCKASGYSFTGYPMNWVRQSHVKNLEWIGVINPYNGGTSYNQKFKGKATLTVDKSSSTAYIELLSLTSDDSAVYYCARGGVRPFAYWGQGTLVTVSA

SEQ ID NO: 2 - protein, 117 aa, synthetic construct
EVQLQQSGPELVKPGASMKISCKASGYSFTGYPMNWVKQTHGKNLEWIGLINPYNGGTSYNQKFKGKATLTVDKSSSTAYMELLSLTSDESAVYYCARGGVRPFDFWGQGTLVTVSA

SEQ ID NO: 3 - protein, 117 aa, synthetic construct
EVQLQQSGPELVKPGASMKISCKASGYSFTGYPMNWVRQSHGKNLEWIGVINSYNGGASYNQKFKGKATLTVDKSSNIVHMELLSLTSEDSAVYYCARGGVRPFAYWGQGTLVTVSA

SEQ ID NO: 4 - protein, 118 aa, synthetic construct
EVQLQQSGPELVKPGASMKISCKASGYSFTGYTMNWVKQSHGENLEWIGVINPYNGGTSYNQKFKGKATLTVDKSFSTAYMEILSLTSEDSAVYYCSRGGGNSWFAYWGQGTLVTVSA

SEQ ID NO: 5 - protein, 118 aa, synthetic construct
EVQLQQSGPELVKPGASMKISCKASGYAFTGYTMNWVKQSHGKNLDWIGVINGYNGGTSYNQKFKGKATLTVDKSSSTAYMELLSLTSEDSAIYYCARGGPTTGFVYWGQGTLVTVSA

SEQ ID NO: 6 - protein, 115 aa, synthetic construct
EVQLQQSGPELVKPGASVKISCKASGYTFTDYYMNWVKQSHGESLEWIGDINPNNGGATYNQKFEGKATLTVDKSSSTAYMELRSLTSEDSAVYYCGQLLGFASWGQGTLVTVSA

SEQ ID NO: 7 - protein, 117 aa, synthetic construct
QVQLVQSGAEVKKPGASVKVSCKASGYTFTGYPMNWVRQAPGQNLEWMGVINPYNGGTSYNQKFKGRVTLTRDKSASTAYMELSSLRSEDTAVYYCARGGVRPFAYWGQGTLVTVSS

SEQ ID NO: 8 - protein, 117 aa, synthetic construct
QVQLVQSGAEVKKPGASVKVSCKASGYTFTGYPMNWVRQAPGKRLEWMGVINPYNGGTSYNQKFKGRATLTVDTSASTAYMELSSLRSEDTAVYYCARGGVRPFAYWGQGTLVTVSS

SEQ ID NO: 9 - protein, 117 aa, synthetic construct
QVQLVQSGAEVKKPGASVKVSCKASGYTFTGYPMNWVRQAPGQNLEWMGVINPYNGGTSYNQKFKGRVTLTVDKSASTAYMELSSLRSEDTAVYYCARGGVRPFAYWGQGTLVTVSS

SEQ ID NO: 10 - protein, 117 aa, synthetic construct
QVQLVQSGAEVKKPGASVKVSCKASGYTFTGYPMNWVRQAPGKNLEWMGVINPYNGGTSYNQKFKGRATLTVDKSASTAYMELSSLRSEDTAVYYCARGGVRPFAYWGQGTLVTVSS

SEQ ID NO: 11 - protein, 117 aa, synthetic construct
QVQLVQSGAEVKKPGASVKVSCKASGYTFTGYPMNWVRQAPGKRLEWMGVINPYSGGTSYNQKFKGRATLTVDTSASTAYMELSSLRSEDTAVYYCARGGVRPFAYWGQGTLVTVSS

SEQ ID NO: 12 - protein, 117 aa, synthetic construct
QVQLVQSGAEVKKPGASVKVSCKASGYTFTGYPMNWVRQAPGKRLEWMGVINPYDGGTSYNQKFKGRATLTVDTSASTAYMELSSLRSEDTAVYYCARGGVRPFAYWGQGTLVTVSS

SEQ ID NO: 13 - protein, 117 aa, synthetic construct
QVQLVQSGAEVKKPGASVKVSCKASGYTFTGYPMNWVRQAPGKRLEWMGVINPYQGGTSYNQKFKGRATLTVDTSASTAYMELSSLRSEDTAVYYCARGGVRPFAYWGQGTLVTVSS

SEQ ID NO: 14 - protein, 117 aa, synthetic construct
QVQLVQSGAEVKKPGASVKVSCKASGYTFTGYPMNWVRQAPGKRLEWMGVINPYNAGTSYNQKFKGRATLTVDTSASTAYMELSSLRSEDTAVYYCARGGVRPFAYWGQGTLVTVSS

SEQ ID NO: 15 - protein, 117 aa, synthetic construct
QVQLVQSGAEVKKPGASVKVSCKASGYTFTGYPMNWVRQAPGKRLEWMGVINPYNVGTSYNQKFKGRATLTVDTSASTAYMELSSLRSEDTAVYYCARGGVRPFAYWGQGTLVTVSS

SEQ ID NO: 16 - protein, 106 aa, synthetic construct
DIQMTQTSSSFSVSLGDRVTITCKASEDIYNRLAWYQQKPGNAPRLLISGATSLETGVPSRFSGSGSGNDYTLSITSLQTEDVATYYCQQYWSTPTFGAGTKLELQ

SEQ ID NO: 17 - protein, 107 aa, synthetic construct
DIVMTQSQKFMSTSVGDRVSVTCKASQNVDTNVAWYQQKPGQSPKALIYSASYRYSGVPDRFTGSGSGTDFTLTISNVQSEDLAEYFCQQYDSYPYTFGGGTKLEIR

SEQ ID NO: 18 - protein, 106 aa, synthetic construct
DIVITQSPAIMSASPGEKVTMTCSARSSVSYMYWYQQKPGSSPRLLIYDTSKLASGVPVRFSGSGSGTSYSLTISRMEAEDAATYFCQQWSSYPPTFGGGTKLEIK

SEQ ID NO: 19 - protein, 106 aa, synthetic construct
DIQMTQTSSYLSVSLGGRVTITCKASDHINNWLAWYQQKPGNAPRLLISGATSLETGVPSRFSGSGSGTDYSLTITSLQTEDVATYYCQQYWSIPTFGGGTRLEIK

SEQ ID NO: 20 - protein, 106 aa, synthetic construct
DIQMTQTSSSFSVSLGDRVTITCKASEDIYNRLAWYQQKPGNAPRLLISGATSLETGVPSRFSGSGSGKDYTLSITSLQTEDVATYYCQQYWSTPTFGAGTKLELK

SEQ ID NO: 21 - protein, 112 aa, synthetic construct
DVVLTQTPLSLPVNIGDQASISCRSTQSLLNSDRFTYLDWYLQRPGQSPQLLIYLVSYRFSGVPDRFSGSGSGTDFTLKISRVEAEDLGLYYCLQSSYLPYTFGGGTKLEIK

SEQ ID NO: 22 - protein, 106 aa, synthetic construct
DIQMTQSPSSLSASVGDRVTITCKASEDIYNRLAWYQQKPGKAPKLLISGATSLETGVPSRFSGSGSGNDFTLTISSLQPEDFATYYCQQYWSTPTFGQGTKLEIK

SEQ ID NO: 23 - protein, 106 aa, synthetic construct
DIQMTQSPSSLSASVGDRVTITCKASEDIYNRLAWYQQKPGNAPKLLISGATSLETGVPSRFSGSGSGNDFTLTISSLQPEDFATYYCQQYWSTPTFGQGTKLEIK

SEQ ID NO: 24 - protein, 106 aa, synthetic construct
DIQMTQSPSSLSASVGDRVTITCKASEDIYNRLAWYQQKPGKAPKLLISGATSLETGVPSRFSGSGSGNDYTLTISSLQPEDFATYYCQQYWSTPTFGQGTKLEIK

SEQ ID NO: 25 - protein, 106 aa, synthetic construct
DIQMTQSPSSLSASVGDRVTITCKASEDIYNRLAWYQQKPGNAPKLLISGATSLETGVPSRFSGSGSGNDYTLTISSLQPEDFATYYCQQYWSTPTFGQGTKLEIK

SEQ ID NO: 26 - protein, 8 aa, synthetic construct
GYSFTGYP

SEQ ID NO: 27 - protein, 8 aa, synthetic construct
INPYNGGT

SEQ ID NO: 28 - protein, 10 aa, synthetic construct
ARGGVRPFAY

SEQ ID NO: 29 - protein, 10 aa, synthetic construct
ARGGVRPFDF

SEQ ID NO: 30 - protein, 8 aa, synthetic construct
INSYNGGA

SEQ ID NO: 31 - protein, 8 aa, synthetic construct
GYSFTGYT

SEQ ID NO: 32 - protein, 11 aa, synthetic construct
SRGGGNSWFAY

SEQ ID NO: 33 - protein, 8 aa, synthetic construct
GYAFTGYT

SEQ ID NO: 34 - protein, 8 aa, synthetic construct
INGYNGGT

SEQ ID NO: 35 - protein, 11 aa, synthetic construct
ARGGPTTGFVY

SEQ ID NO: 36 - protein, 8 aa, synthetic construct
GYTFTDYY

SEQ ID NO: 37 - protein, 8 aa, synthetic construct
INPNNGGA

SEQ ID NO: 38 - protein, 8 aa, synthetic construct
GQLLGFAS

SEQ ID NO: 39 - protein, 8 aa, synthetic construct
GYTFTGYP

SEQ ID NO: 40 - protein, 8 aa, synthetic construct
INPYSGGT

SEQ ID NO: 41 - protein, 8 aa, synthetic construct
INPYDGGT

SEQ ID NO: 42 - protein, 8 aa, synthetic construct
INPYQGGT

SEQ ID NO: 43 - protein, 8 aa, synthetic construct
INPYNAGT

SEQ ID NO: 44 - protein, 8 aa, synthetic construct
INPYNVGT

SEQ ID NO: 45 - protein, 6 aa, synthetic construct
EDIYNR

SEQ ID NO: 46 - protein, 8 aa, synthetic construct
QQYWSTPT

SEQ ID NO: 47 - protein, 6 aa, synthetic construct
QNVDTN

SEQ ID NO: 48 - protein, 9 aa, synthetic construct
QQYDSYPYT

SEQ ID NO: 49 - protein, 5 aa, synthetic construct
SSVSY

SEQ ID NO: 50 - protein, 9 aa, synthetic construct
QQWSSYPPT

SEQ ID NO: 51 - protein, 6 aa, synthetic construct
DHINNW

SEQ ID NO: 52 - protein, 8 aa, synthetic construct
QQYWSIPT

SEQ ID NO: 53 - protein, 11 aa, synthetic construct
QSLLNSDRFTY

SEQ ID NO: 54 - protein, 9 aa, synthetic construct
LQSSYLPYT

SEQ ID NO: 55 - protein, 25 aa, synthetic construct
EVQLQQSGPELVKPGASMKISCKAS

SEQ ID NO: 56 - protein, 25 aa, synthetic construct
EVQLQQSGPELVKPGASVKISCKAS

SEQ ID NO: 57 - protein, 25 aa, synthetic construct [sequence omitted]

SEQ ID NO: 58 - protein, 17 aa, synthetic construct
MNWVKQSHGENLEWIGV

SEQ ID NO: 59 - protein, 17 aa, synthetic construct
MNWVKQSHGESLEWIGD

SEQ ID NO: 60 - protein, 17 aa, synthetic construct
MNWVKQSHGKNLDWIGV

SEQ ID NO: 61 - protein, 17 aa, synthetic construct
MNWVKQTHGKNLEWIGL

SEQ ID NO: 62 - protein, 17 aa, synthetic construct
MNWVRQAPGKNLEWMGV

SEQ ID NO: 63 - protein, 17 aa, synthetic construct
MNWVRQAPGKRLEWMGV

SEQ ID NO: 64 - protein, 17 aa, synthetic construct
MNWVRQAPGQNLEWMGV

SEQ ID NO: 65 - protein, 17 aa, synthetic construct
MNWVRQSHGKNLEWIGV

SEQ ID NO: 66 - protein, 17 aa, synthetic construct
MNWVRQSHVKNLEWIGV

SEQ ID NO: 67 - protein, 38 aa, synthetic construct
SYNQKFKGRVTLTVDKSASTAYMELSSLRSEDTAVYYC

SEQ ID NO: 68 - protein, 38 aa, synthetic construct
SYNQKFKGKATLTVDKSFSTAYMEILSLTSEDSAVYYC

SEQ ID NO: 69 - protein, 38 aa, synthetic construct
SYNQKFKGKATLTVDKSSNIVHMELLSLTSEDSAVYYC

SEQ ID NO: 70 - protein, 38 aa, synthetic construct
SYNQKFKGKATLTVDKSSSTAYIELLSLTSDDSAVYYC

SEQ ID NO: 71 - protein, 38 aa, synthetic construct
SYNQKFKGKATLTVDKSSSTAYMELLSLTSDESAVYYC

SEQ ID NO: 72 - protein, 38 aa, synthetic construct
SYNQKFKGKATLTVDKSSSTAYMELLSLTSEDSAIYYC

SEQ ID NO: 73 - protein, 38 aa, synthetic construct
SYNQKFKGRATLTVDKSASTAYMELSSLRSEDTAVYYC

SEQ ID NO: 74 - protein, 38 aa, synthetic construct
SYNQKFKGRATLTVDTSASTAYMELSSLRSEDTAVYYC

SEQ ID NO: 75 - protein, 38 aa, synthetic construct
SYNQKFKGRVTLTRDKSASTAYMELSSLRSEDTAVYYC

SEQ ID NO: 76 - protein, 38 aa, synthetic construct
TYNQKFEGKATLTVDKSSSTAYMELRSLTSEDSAVYYC

SEQ ID NO: 77 - protein, 11 aa, synthetic construct
WGQGTLVTVSA

SEQ ID NO: 78 - protein, 11 aa, synthetic construct
WGQGTLVTVSS

SEQ ID NO: 79 - protein, 26 aa, synthetic construct [sequence omitted]

SEQ ID NO: 80 - protein, 26 aa, synthetic construct
DIQMTQTSSSFSVSLGDRVTITCKAS

SEQ ID NO: 81 - protein, 26 aa, synthetic construct
DIQMTQTSSYLSVSLGGRVTITCKAS

SEQ ID NO: 82 - protein, 26 aa, synthetic construct
DIVITQSPAIMSASPGEKVTMTCSAR

SEQ ID NO: 83 - protein, 26 aa, synthetic construct
DIVMTQSQKFMSTSVGDRVSVTCKAS

SEQ ID NO: 84 - protein, 26 aa, synthetic construct
DVVLTQTPLSLPVNIGDQASISCRST

SEQ ID NO: 85 - protein, 17 aa, synthetic construct
LAWYQQKPGKAPKLLIS

SEQ ID NO: 86 - protein, 17 aa, synthetic construct
LAWYQQKPGNAPKLLIS

SEQ ID NO: 87 - protein, 17 aa, synthetic construct
LAWYQQKPGNAPRLLIS

SEQ ID NO: 88 - protein, 17 aa, synthetic construct
LDWYLQRPGQSPQLLIY

SEQ ID NO: 89 - protein, 17 aa, synthetic construct
MYWYQQKPGSSPRLLIY

SEQ ID NO: 90 - protein, 17 aa, synthetic construct
VAWYQQKPGQSPKALIY

SEQ ID NO: 91 - protein, 36 aa, synthetic construct
KLASGVPVRFSGSGSGTSYSLTISRMEAEDAATYFC

SEQ ID NO: 92 - protein, 36 aa, synthetic construct
SLETGVPSRFSGSGSGKDYTLSITSLQTEDVATYYC

SEQ ID NO: 93 - protein, 36 aa, synthetic construct
SLETGVPSRFSGSGSGNDFTLTISSLQPEDFATYYC

SEQ ID NO: 94 - protein, 36 aa, synthetic construct
SLETGVPSRFSGSGSGNDYTLSITSLQTEDVATYYC

SEQ ID NO: 95 - protein, 36 aa, synthetic construct
SLETGVPSRFSGSGSGNDYTLTISSLQPEDFATYYC

SEQ ID NO: 96 - protein, 36 aa, synthetic construct
SLETGVPSRFSGSGSGTDYSLTITSLQTEDVATYYC

SEQ ID NO: 97 - protein, 36 aa, synthetic construct
YRFSGVPDRFSGSGSGTDFTLKISRVEAEDLGLYYC

SEQ ID NO: 98 - protein, 36 aa, synthetic construct
YRYSGVPDRFTGSGSGTDFTLTISNVQSEDLAEYFC

SEQ ID NO: 99 - protein, 10 aa, synthetic construct
FGAGTKLELK

SEQ ID NO: 100 - protein, 10 aa, synthetic construct
FGGGTKLEIK

SEQ ID NO: 101 - protein, 10 aa, synthetic construct
FGGGTKLEIR

SEQ ID NO: 102 - protein, 10 aa, synthetic construct
FGGGTRLEIK

SEQ ID NO: 103 - protein, 10 aa, synthetic construct
FGQGTKLEIK

SEQ ID NO: 104 - DNA, 21 bp, synthetic construct
  source 1..21: mol_type = other DNA
ttacgccgctgacattgtgtt

SEQ ID NO: 105 - DNA, 19 bp, synthetic construct
  source 1..19: mol_type = other DNA
accagcccttcgagaaagc

SEQ ID NO: 106 - DNA, 22 bp, synthetic construct
  source 1..22: mol_type = other DNA
ggagagtgtctgcggatacttc

SEQ ID NO: 107 - DNA, 23 bp, synthetic construct
  source 1..23: mol_type = other DNA
gcaggtagtgatgtgcaagagtc

SEQ ID NO: 108 - DNA, 24 bp, synthetic construct
  source 1..24: mol_type = other DNA
gagcggtcggcgtcccccaacttc

SEQ ID NO: 109 - DNA, 24 bp, synthetic construct
  source 1..24: mol_type = other DNA
gcgcgtgcagccccggacatctaa